European Patent Application EP 4 502 156 A1, published February 5, 2025. Title: Genome-modified silkworm producing chimeric silk thread. Applicant: 国立研究開発法人農業・食品産業技術総合研究機構. The sequence listing filed with the application follows.

SEQUENCE LISTING (34 sequences)

SEQ ID NO: 1 - protein, 34 aa, synthetic construct
  REGION 1..34: note = synthetic
  REGION 12..13: note = misc_feature - Xaa can be any naturally occurring amino acid
LTPDQVVAIASXXGGKQALETVQRLLPVLCQDHG

SEQ ID NO: 2 - DNA, 677 bp, Bombyx mori
  source 1..677: mol_type = unassigned DNA
gcttgatgcgcgttaccatatatggtgacaaaaactgagtcagcccgcgattggtggaaaaacaaactggagccgatactgtgtaaattgtgataacggctcttttatatagtttatcctcacgagtcggttctcatttactaaggtgtgctcgaacagtgcgcattcgcatctacgtacttgtcacttatttaataatactatgtaagttttaattttaaaattgcgaaagaaaaaaaaacatatttatttatttgtaaaatttgaatttcgaaggttctccgtccctttacctttaagtattacatatgtttgagtgttttttttttttaataatacgctaatgataacgtgttatgttacataattgttgcataactagtgaagtgaaattttttataaaaaaaaaaacagttttcggaattagtgtactgcagatgttaataaacactactaaataagaaataagtttattggacgcacatttcaaagtgtccactcgcatcgatcaattcggaaacagaaattgggaacagtgaattatgaatcttatacagttttctttaacgtcactaaatagatggacgcaaataaatttgtcgtttacttagtataatgtatggaatgagaatgtagtttgaattgttttttttcttttcttgcagactaattcaaga

SEQ ID NO: 3 - protein, 22 aa, Eumeta japonica
AAAAAAAAAEAAAAAAAAAAAA

SEQ ID NO: 4 - protein, 19 aa, Eumeta japonica
AAAAAAAAAQAAAAAAAAA

SEQ ID NO: 5 - protein, 7 aa, Eumeta japonica
YGSALNS

SEQ ID NO: 6 - protein, 5 aa, Eumeta japonica
SALNS

SEQ ID NO: 7 - protein, 6 aa, Eumeta japonica
TSVVYV

SEQ ID NO: 8 - protein, 151 aa, Eumeta japonica
AAAAAAAAAQAAAAAAAAAGSGAGAGRVGAYGPYGGLASAGAGGAGGAGGAGGYGGASVVYVGGGGAGAGAGSGAGAGSGAGAGAGSGAGAGGAGAAAGAGAGAGSGAGSGSGAGAGAGSGAGAGSGAGAGAGAGSGAAGGAGAGAGAGAG

SEQ ID NO: 9 - protein, 178 aa, Eumeta japonica
AAAAAAAAAEAAAAAAAAAAAAGSGAGAGGAGGYGAGAGAGAGAGAGGAAGAGGAGGAGGAGGYGGASAGAGGAGGAGGAGGYGGAGVVYVSAGGAGAGAGSGAGAGSGAGAGAGSGAGAGGAGAAAGAGAGAGSGAGSGSGAGAGAGSGAGAGSGAGAGAGAGSGAAGGAGAGAGAG

SEQ ID NO: 10 - protein, 133 aa, Eumeta japonica
AAAAAAAAAEAAAAAAAAAAAAGSGAGAGGAGGYGAGAGAGAGAGAGGASGGYGSYGSGVAAGAGAGAGVGGSRGAGVGAGVGAGYGSALNSGAGAGAGAGAGAGGAAGAGAGAGAGAGSGAAGGAGAGAGAG

SEQ ID NO: 11 - protein, 153 aa, Eumeta japonica
AAAAAAAAAEAAAAAAAAAAAAGGAGGYGAGAGAGAGAGAGTSAGAGGAGGAGGAGGYGGAGVVYVSAGGAGAGAGSGAGAGSGAGAGAGSGAGAGGAGAAAGAGAGAGSGAGSGSGAGAGAGSGAGAGSGAGAGAGAGSGAAGGAGAGAGAG

SEQ ID NO: 12 - protein, 128 aa, Eumeta japonica
AAAAAAAAAEAAAAAAAAAAAAGGAGGYGAGAGAGAGAGAGTSVVYVSAGGAGAGAGSGAGAGSGAGAGAGSGAGAGGAGAAAGAGAGAGSGAGSGSGAGAGAGSGAVAGSGAGSGAAGGAGAGAGAG

SEQ ID NO: 13 - protein, 153 aa, Eumeta japonica
AAAAAAAAAEAAAAAAAAAAAAGSGAGAGGAGGYGAGAGAGAGAGVGGAGGAGGAGGAGGAGGYGGAGVVYVSAGGAGAGAGSGAGAGSGAGAGAGSGAGAGGAGAAAGAGAGAGSGAGSGSGAGAGAGSGAVAGSGAGSGAAGGAGAGAGAG

SEQ ID NO: 14 - protein, 123 aa, Eumeta japonica
AAAAAAAAAEAAAAAAAAAAAAGSGAGAGGAGGYGAGAGAGAGAGAGGASGGYGSYGSGVAAGAGAGAGVGGSRGAGVGAGVGAGYGSALNSGAGAGAGAGAGAGGAAGAGAGAGAGAGAGAG

SEQ ID NO: 15 - protein, 153 aa, Eumeta japonica
AAAAAAAAAEAAAAAAAAAAAAGSGAGAGGAGGYGAGAGAGAGAGAGGAAGAGGAGGAGGAGGYGGASVVYVSAGGAGAGAGSGAGAGSGAGAGAGSGAGAGGAGAAAGAGAGAGSGAGSGSGAGAGAGSGAVAGSGAGSGAAGGAGAGAGAG

SEQ ID NO: 16 - protein, 161 aa, Eumeta japonica
AAAAAAAAAEAAAAAAAAAAAAGSGAGAGGAGGYGAGAGAGAGAGAGGAAGAGGAGGAGGAGGYGGTSVVYVGGGGAGAGAGSGAGAGSGAGAGAGSGAGAGGAGAAAGAGAGAGSGAGSGSGAGAGAGSGAGAGSGAGAGAGAGSGAAGGAGAGAGAGAG

SEQ ID NO: 17 - DNA, 453 bp, Eumeta japonica
  source 1..453: mol_type = unassigned DNA
gctgcagccgccgctgcggcagcagcacaagcagcagccgcagctgctgccgccgcaggtagtggcgctggtgctggacgagtcggagcttacggaccctacggaggtttagcaagcgctggtgctggtggtgctggcggagccggtggtgcaggtggatacggtggtgcaagtgtcgtctacgtaggtggcggaggagccggagcaggtgccggttcaggcgccggtgctggatcgggtgccggagcaggagctggatcaggtgcaggagcaggtggagcaggagccgcagccggagctggtgctggtgctggttcaggtgcaggatccggttcaggtgcgggcgctggagcaggttccggagcaggagcaggttccggtgctggtgcaggagcaggagctggctcaggtgcagcaggtggagcaggagcaggagctggcgctggcgctggc

SEQ ID NO: 18 - DNA, 534 bp, Eumeta japonica
  source 1..534: mol_type = unassigned DNA
gctgcagccgcagccgcagcagcagcagaagcggcagccgcagctgccgccgccgctgccgccgcaggtagtggagcaggcgctggaggagccggaggctacggagcgggagctggagcaggtgccggtgcaggtgctggcggcgctgctggtgctggtggtgctggcggagccggtggtgcaggtggatacggtggtgctagcgcgggtgcgggtggcgcgggtggcgcgggtggcgcgggtggctacggtggcgcgggtgtggtttatgttagcgcgggtggcgcgggcgcgggtgcgggtagcggtgcgggtgcgggcagcggtgccggcgcgggcgcgggcagcggcgcgggagcgggtggcgcgggcgctgcggcgggtgcgggcgcgggtgcgggcagcggagcgggatccggtagcggcgctggcgctggtgcgggtagcggagctggcgcgggcagcggtgcgggtgcgggtgcgggcgcgggtagcggtgcggcgggtggcgcgggagcaggcgcgggtgcgggt

SEQ ID NO: 19 - DNA, 399 bp, Eumeta japonica
  source 1..399: mol_type = unassigned DNA
gccgctgccgccgcggcggcggcggcggaggcagctgccgcagcagctgccgcagcggcggcggcgggtagcggtgcgggcgcgggtggcgcgggtggctacggggctggcgctggtgctggtgctggtgctggcgcgggtggcgcgagcggtggctacggtagctatggcagcggtgtggcggcgggtgctggcgcgggcgcgggtgttggtggcagccgtggcgcgggtgtgggtgcgggtgttggtgcgggttatggcagcgcgctgaatagcggcgctggagcaggtgctggtgccggcgctggcgcgggtggcgcggctggcgctggtgccggtgctggtgcaggagctggcagcggagctgcgggtggcgccggagctggagctggcgcggga

SEQ ID NO: 20 - DNA, 459 bp, Eumeta japonica
  source 1..459: mol_type = unassigned DNA
gctgccgccgctgccgcagctgcggcggaagcagctgccgccgctgctgctgctgctgctgccgcgggtggcgcgggtggctacggagctggagccggcgcaggcgctggtgccggcgcgggtactagcgcgggtgcgggtggcgcgggtggcgcgggtggcgcgggtggctacggtggcgcgggtgtggtttatgttagcgcgggtggcgcgggcgcgggtgcgggtagcggtgcgggtgcgggcagcggtgccggcgcgggcgcgggcagcggcgcgggagcgggtggcgcgggcgctgcggcgggtgcgggcgcgggtgcgggcagcggagcgggatccggtagcggcgctggcgctggtgcgggtagcggagctggcgcgggcagcggtgcgggtgcgggtgcgggcgcgggtagcggtgcggcgggtggcgcgggagcaggcgcgggtgcgggt

SEQ ID NO: 21 - DNA, 384 bp, Eumeta japonica
  source 1..384: mol_type = unassigned DNA
gctgccgccgctgccgcagctgcggcggaagcagctgccgccgctgctgctgctgctgctgccgcgggtggcgcgggtggctacggagctggagccggcgcaggcgctggtgccggcgcgggtactagcgtcgtctacgtaagtgctggaggagccggagcaggtgccggttcaggcgccggtgctggatcgggtgccggagcaggagctggatcaggtgcaggagcaggtggagcaggagccgcagccggagctggtgctggtgctggttcaggtgcaggatccggttcaggtgcgggcgctggagcaggttccggagcagtagcaggttccggtgctggttcaggtgcagcaggtggagcaggagctggcgctggcgctggc

SEQ ID NO: 22 - DNA, 459 bp, Eumeta japonica
  source 1..459: mol_type = unassigned DNA
gctgcagccgcagccgcagcagcagcagaagcggcagccgcagctgccgccgccgctgccgccgcaggtagtggagcaggcgctggaggagccggaggctacggagcgggagctggagcaggtgccggagcaggtgttggcggcgctggtggtgctggtggtgctggcggagccggtggtgcaggtggatacggtggtgcaggcgtcgtctacgtaagtgctggaggagccggagcaggtgccggttcaggcgccggtgctggatcgggtgccggagcaggagctggatcaggtgcaggagcaggtggagcaggagccgcagccggagctggtgctggtgctggttcaggtgcaggatccggttcaggtgcgggcgctggagcaggttccggagcagtagcaggttccggtgctggttcaggtgcagcaggtggagcaggagctggcgctggcgctggc

SEQ ID NO: 23 - DNA, 369 bp, Eumeta japonica
  source 1..369: mol_type = unassigned DNA
gctgcagccgcagccgcagcagcagcagaagcggcagccgcagctgccgccgccgctgccgccgcaggtagtggagcaggcgctggaggagccggaggctacggagcgggagctggagcaggtgccggtgcaggtgctggcggcgcatctggaggctacggttcttacggatcgggagttgcagcaggtgccggtgcaggagctggtgttggtggtagcaggggagcaggtgttggcgctggtgttggtgctggttatggctccgcattgaattcaggagccggtgccggagcaggtgctggtgctggagctggtggtgctgcaggagctggtgctggtgcaggagcaggagctggcgctggagctgga

SEQ ID NO: 24 - DNA, 459 bp, Eumeta japonica
  source 1..459: mol_type = unassigned DNA
gctgcagccgcagccgcagcagcagcagaagcggcagccgcagctgccgccgccgctgccgccgcaggtagtggagcaggcgctggaggagccggaggctacggagcgggagctggagcaggtgccggtgcaggtgctggcggcgctgctggtgctggtggtgctggcggagccggtggtgcaggtggatacggtggtgctagcgtcgtctacgtaagtgctggaggagccggagcaggtgccggttcaggcgccggtgctggatcgggtgccggagcaggagctggatcaggtgcaggagcaggtggagcaggagccgcagccggagctggtgctggtgctggttcaggtgcaggatccggttcaggtgcgggcgctggagcaggttccggagcagtagcaggttccggtgctggttcaggtgcagcaggtggagcaggagctggcgctggcgctggc

SEQ ID NO: 25 - DNA, 483 bp, Eumeta japonica
  source 1..483: mol_type = unassigned DNA
gctgcagccgcagccgcagcagcagcagaagcggcagccgcagctgccgccgccgctgccgccgcaggtagtggagcaggcgctggaggagccggaggctacggagcgggagctggagcaggtgccggtgcaggtgctggcggcgctgctggtgctggtggtgctggcggagccggtggtgcaggtggatacggtggtactagcgtcgtctacgtaggtggcggaggagccggagcaggtgccggttcaggcgccggtgctggatcgggtgccggagcaggagctggatcaggtgctggagcaggtggagcaggagccgcagccggagctggtgctggtgctggttcaggtgcaggatccggttcaggtgcgggcgctggagcaggttccggagcaggagcaggttccggtgctggtgcaggagcaggagctggttcaggtgcagcaggtggagcaggagcaggagctggcgctggcgctggc

SEQ ID NO: 26 - protein, 753 aa, synthetic construct
  REGION 1..753: note = synthetic
MAKADWYEDWKKNQGSFRETDLADTDEYQTDSNGTMFEKKTTRKKFEKDGSTMVNSDSGEDKIVRTFVVETDASGHEVIYEEDVVIKKVPGKRKKVSQANAKASAIAASVGAGVGAASVAGAGTGAGSGAAGGAGAGADAGAAAAAAAAAQAAAAAAAAAGSGAGAGRVGAYGPYGGLASAGAGGAGGAGGAGGYGGASVVYVGGGGAGAGAGSGAGAGSGAGAGAGSGAGAGGAGAAAGAGAGAGSGAGSGSGAGAGAGSGAGAGSGAGAGAGAGSGAAGGAGAGAGAGAGAAAAAAAAAEAAAAAAAAAAAAGSGAGAGGAGGYGAGAGAGAGAGAGGAAGAGGAGGAGGAGGYGGASVVYVSAGGAGAGAGSGAGAGSGAGAGAGSGAGAGGAGAAAGAGAGAGSGAGSGSGAGAGAGSGAVAGSGAGSGAAGGAGAGAGAGAAAAAAAAAEAAAAAAAAAAAAGSGAGAGGAGGYGAGAGAGAGAGVGGAGGAGGAGGAGGAGGYGGAGVVYVSAGGAGAGAGSGAGAGSGAGAGAGSGAGAGGAGAAAGAGAGAGSGAGSGSGAGAGAGSGAVAGSGAGSGAAGGAGAGAGAGAAAAAAAAAEAAAAAAAAAAAAGSGAGAGGAGGYGAGAGAGAGAGAGGASGGYGSYGSGVAAGAGAGAGVGGSRGAGVGAGVGAGYGSALNSGAGAGAGAGAGAGGAAGAGAGAGAGAGAGAGFASYGRPGVRGCQLSRKYLLVKVGLRSTCSDC

SEQ ID NO: 27 - protein, 1865 aa, Eumeta japonica
MAKADWYEDWKKNQGSFRETDLADTDEYQTDSNGTMFEKKTTRKKFEKDGSTMVNSDSGEDKIVRTFVVETDASGHEVIYEEDVVIKKVPGKRKKVSQANAKASAIAASVGAGVGAASVAGAGTGAGSGAAGGAGAGADAGAAAAAAAAAQAAAAAAAAAGSGAGAGRVGAYGPYGGLASAGAGGAGGAGGAGGYGGASVVYVGGGGAGAGAGSGAGAGSGAGAGAGSGAGAGGAGAAAGAGAGAGSGAGSGSGAGAGAGSGAGAGSGAGAGAGAGSGAAGGAGAGAGAGAGAAAAAAAAAEAAAAAAAAAAAAGSGAGAGGAGGYGAGAGAGAGAGAGGAAGAGGAGGAGGAGGYGGASAGAGGAGGAGGAGGYGGAGVVYVSAGGAGAGAGSGAGAGSGAGAGAGSGAGAGGAGAAAGAGAGAGSGAGSGSGAGAGAGSGAGAGSGAGAGAGAGSGAAGGAGAGAGAGAAAAAAAAAEAAAAAAAAAAAAGSGAGAGGAGGYGAGAGAGAGAGAGGASGGYGSYGSGVAAGAGAGAGVGGSRGAGVGAGVGAGYGSALNSGAGAGAGAGAGAGGAAGAGAGAGAGAGSGAAGGAGAGAGAGAAAAAAAAAEAAAAAAAAAAAAGGAGGYGAGAGAGAGAGAGTSAGAGGAGGAGGAGGYGGAGVVYVSAGGAGAGAGSGAGAGSGAGAGAGSGAGAGGAGAAAGAGAGAGSGAGSGSGAGAGAGSGAGAGSGAGAGAGAGSGAAGGAGAGAGAGAAAAAAAAAEAAAAAAAAAAAAGSGAGAGGAGGYGAGAGAGAGAGAGGASGGYGSYGSGVAAGAGAGAGVGGSRGAGVGAGVGAGYGSALNSGAGAGAGAGAGAGGAAGAGAGAGAGAGSGAAGGAGAGAGAGAAAAAAAAAEAAAAAAAAAAAAGGAGGYGAGAGAGAGAGAGTSAGAGGAGGAGGAGGYGGAGVVYVSAGGAGAGAGSGAGAGSGAGAGAGSGAGAGGAGAAAGAGAGAGSGAGSGSGAGAGAGSGAGAGSGAGAGAGAGSGAAGGAGAGAGAGAAAAAAAAAEAAAAAAAAAAAAGSGAGAGGAGGYGAGAGAGAGAGAGGASGGYGSYGSGVAAGAGAGAGVGGSRGAGVGAGVGAGYGSALNSGAGAGAGAGAGAGGAAGAGAGAGAGAGSGAAGGAGAGAGAGAAAAAAAAAEAAAAAAAAAAAAGGAGGYGAGAGAGAGAGAGTSAGAGGAGGAGGAGGYGGAGVVYVSAGGAGAGAGSGAGAGSGAGAGAGSGAGAGGAGAAAGAGAGAGSGAGSGSGAGAGAGSGAGAGSGAGAGAGAGSGAAGGAGAGAGAGAAAAAAAAAEAAAAAAAAAAAAGSGAGAGGAGGYGAGAGAGAGAGAGGASGGYGSYGSGVAAGAGAGAGVGGSRGAGVGAGVGAGYGSALNSGAGAGAGAGAGAGGAAGAGAGAGAGAGSGAAGGAGAGAGAGAAAAAAAAAEAAAAAAAAAAAAGGAGGYGAGAGAGAGAGAGTSVVYVSAGGAGAGAGSGAGAGSGAGAGAGSGAGAGGAGAAAGAGAGAGSGAGSGSGAGAGAGSGAVAGSGAGSGAAGGAGAGAGAGAAAAAAAAAEAAAAAAAAAAAAGSGAGAGGAGGYGAGAGAGAGAGVGGAGGAGGAGGAGGAGGYGGAGVVYVSAGGAGAGAGSGAGAGSGAGAGAGSGAGAGGAGAAAGAGAGAGSGAGSGSGAGAGAGSGAVAGSGAGSGAAGGAGAGAGAGAAAAAAAAAEAAAAAAAAAAAAGSGAGAGGAGGYGAGAGAGAGAGAGGASGGYGSYGSGVAAGAGAGAGVGGSRGAGVGAGVGAGYGSALNSGAGAGAGAGAGAGGAAGAGAGAGAGAGAGAG

SEQ ID NO: 28 - DNA, 5595 bp, synthetic construct
  misc_feature 1..5595: note = synthetic
  source 1..5595: mol_type = other DNA
atggcgaaggcggattggtatgaagattggaaaaaaaaccaaggttcatttagagaaacagacttagcagacactgacgaatatcaaacagatagtaatggtacaatgtttgaaaaaaaaacaacaagaaaaaagttcgaaaaagatggaagtactatggtaaacagtgattccggagaagataaaattgtacgaactttcgtcgtggaaactgacgcatcaggacatgaagttatttatgaagaagatgtagtcattaaaaaagttccaggtaaacggaagaaagtttcacaggcaaatgctaaagctagtgctatagcagccagtgtaggtgcgggcgttggagcagcttccgttgctggtgcaggaacaggagctggctcaggtgcagctggtggagcaggagcaggtgctgacgctggcgctgcagccgccgctgcggcagcagcacaagcagcagccgcagctgctgccgccgcaggtagtggcgctggtgctggacgagtcggagcttacggaccctacggaggtttagcaagcgctggtgctggtggtgctggcggagccggtggtgcaggtggatacggtggtgcaagtgtcgtctacgtaggtggcggaggagccggagcaggtgccggttcaggcgccggtgctggatcgggtgccggagcaggagctggatcaggtgcaggagcaggtggagcaggagccgcagccggagctggtgctggtgctggttcaggtgcaggatccggttcaggtgcgggcgctggagcaggttccggagcaggagcaggttccggtgctggtgcaggagcaggagctggctcaggtgcagcaggtggagcaggagcaggagctggcgctggcgctggcgctgcagccgcagccgcagcagcagcagaagcggcagccgcagctgccgccgccgctgccgccgcaggtagtggagcaggcgctggaggagccggaggctacggagcgggagctggagcaggtgccggtgcaggtgctggcggcgctgctggtgctggtggtgctggcggagccggtggtgcaggtggatacggtggtgctagcgcgggtgcgggtggcgcgggtggcgcgggtggcgcgggtggctacggtggcgcgggtgtggtttatgttagcgcgggtggcgcgggcgcgggtgcgggtagcggtgcgggtgcgggcagcggtgccggcgcgggcgcgggcagcggcgcgggagcgggtggcgcgggcgctgcggcgggtgcgggcgcgggtgcgggcagcggagcgggatccggtagcggcgctggcgctggtgcgggtagcggagctggcgcgggcagcggtgcgggtgcgggtgcgggcgcgggtagcggtgcggcgggtggcgcgggagcaggcgcgggtgcgggtgccgctgccgccgcggcggcggcggcggaggcagctgccgcagcagctgccgcagcggcggcggcgggtagcggtgcgggcgcgggtggcgcgggtggctacggggctggcgctggtgctggtgctggtgctggcgcgggtggcgcgagcggtggctacggtagctatggcagcggtgtggcggcgggtgctggcgcgggcgcgggtgttggtggcagccgtggcgcgggtgtgggtgcgggtgttggtgcgggttatggcagcgcgctgaatagcggcgctggagcaggtgctggtgccggcgctggcgcgggtggcgcggctggcgctggtgccggtgctggtgcaggagctggcagcggagctgcgggtggcgccggagctggagctggcgcgggagctgccgccgctgccgcagctgcggcggaagcagctgccgccgctgctgctgctgctgctgccgcgggtggcgcgggtggctacggagctggagccggcgcaggcgctggtgccggcgcgggtactagcgcgggtgcgggtggcgcgggtggcgcgggtggcgcgggtggctacggtggcgcgggtgtggtttatgttagcgcgggtggcgcgggcgcgggtgcgggtagcggtgcgggtgcgggcagcggtgccggcgcgggcgcgggcagcggcgcgggagcgggtggcgcgggcgctgcggcgggtgcgggcgcgggtgcgggcagcggagcgggatccggtagcggcgctggcgctggtgcgggtagcggagctggcgcgggcagcggtgcgggtgcgggtgcgggcgcgggtagcggtgcggcgggtggcgcgggagcaggcgcgggtgcgggtgccgctgccgccgcggcggcggcggcggaggcagctgccgcagcagctgccgcagcggcggcggcgggtagcggtgcgggcgcgggtggcgcgggtggctacggggctggcgctggtgctggtgctggtgctggcgcgggtggcgcgagcggtggctacggtagctatggcagcggtgtggcggcgggtgctggcgcgggcgcgggtgttggtggcagccgtggcgcgggtgtgggtgcgggtgttggtgcgggttatggcagcgcgctgaatagcggcgctggagcaggtgctggtgccggcgctggcgcgggtggcgcggctggcgctggtgccggtgctggtgcaggagctggcagcggagctgcgggtggcgccggagctggagctggcgcgggagctgccgccgctgccgcagctgcggcggaagcagctgccgccgctgctgctgctgctgctgccgcgggtggcgcgggtggctacggagctggagccggcgcaggcgctggtgccggcgcgggtactagcgcgggtgcgggtggcgcgggtggcgcgggtggcgcgggtggctacggtggcgcgggtgtggtttatgttagcgcgggtggcgcgggcgcgggtgcgggtagcggtgcgggtgcgggcagcggtgccggcgcgggcgcgggcagcggcgcgggagcgggtggcgcgggcgctgcggcgggtgcgggcgcgggtgcgggcagcggagcgggatccggtagcggcgctggcgctggtgcgggtagcggagctggcgcgggcagcggtgcgggtgcgggtgcgggcgcgggtagcggtgcggcgggtggcgcgggagcaggcgcgggtgcgggtgccgctgccgccgcggcggcggcggcggaggcagctgccgcagcagctgccgcagcggcggcggcgggtagcggtgcgggcgcgggtggcgcgggtggctacggggctggcgctggtgctggtgctggtgctggcgcgggtggcgcgagcggtggctacggtagctatggcagcggtgtggcggcgggtgctggcgcgggcgcgggtgttggtggcagccgtggcgcgggtgtgggtgcgggtgttggtgcgggttatggcagcgcgctgaatagcggcgctggagcaggtgctggtgccggcgctggcgcgggtggcgcggctggcgctggtgccggtgctggtgcaggagctggcagcggagctgcgggtggcgccggagctggagctggcgcgggagctgccgccgctgccgcagctgcggcggaagcagctgccgccgctgctgctgctgctgctgccgcgggtggcgcgggtggctacggagctggagccggcgcaggcgctggtgccggcgcgggtactagcgcgggtgcgggtggcgcgggtggcgcgggtggcgcgggtggctacggtggcgcgggtgtggtttatgttagcgcgggtggcgcgggcgcgggtgcgggtagcggtgcgggtgcgggcagcggtgccggcgcgggcgcgggcagcggcgcgggagcgggtggcgcgggcgctgcggcgggtgcgggcgcgggtgcgggcagcggagcgggatccggtagcggcgctggcgctggtgcgggtagcggagctggcgcgggcagcggtgcgggtgcgggtgcgggcgcgggtagcggtgcggcgggtggcgcgggagcaggcgcgggtgcgggtgccgctgccgccgcggcggcggcggcggaggcagctgccgcagcagctgccgcagcggcggcggcgggtagcggtgcgggcgcgggtggcgcgggtggctacggggctggcgctggtgctggtgctggtgctggcgcgggtggcgcgagcggtggctacggtagctatggcagcggtgtggcggcgggtgctggcgcgggcgcgggtgttggtggcagccgtggcgcgggtgtgggtgcgggtgttggtgcgggttatggcagcgcgctgaatagcggcgctggagcaggtgctggtgccggcgctggcgcgggtggcgcggctggcgctggtgccggtgctggtgcaggagctggcagcggagctgcgggtggcgccggagctggagctggcgcgggagctgccgccgctgccgcagctgcggcggaagcagctgccgccgctgctgctgctgctgctgccgcgggtggcgcgggtggctacggagctggagccggcgcaggcgctggtgccggcgcgggtactagcgtcgtctacgtaagtgctggaggagccggagcaggtgccggttcaggcgccggtgctggatcgggtgccggagcaggagctggatcaggtgcaggagcaggtggagcaggagccgcagccggagctggtgctggtgctggttcaggtgcaggatccggttcaggtgcgggcgctggagcaggttccggagcagtagcaggttccggtgctggttcaggtgcagcaggtggagcaggagctggcgctggcgctggcgctgcagccgcagccgcagcagcagcagaagcggcagccgcagctgccgccgccgctgccgccgcaggtagtggagcaggcgctggaggagccggaggctacggagcgggagctggagcaggtgccggagcaggtgttggcggcgctggtggtgctggtggtgctggcggagccggtggtgcaggtggatacggtggtgcaggcgtcgtctacgtaagtgctggaggagccggagcaggtgccggttcaggcgccggtgctggatcgggtgccggagcaggagctggatcaggtgcaggagcaggtggagcaggagccgcagccggagctggtgctggtgctggttcaggtgcaggatccggttcaggtgcgggcgctggagcaggttccggagcagtagcaggttccggtgctggttcaggtgcagcaggtggagcaggagctggcgctggcgctggcgctgcagccgcagccgcagcagcagcagaagcggcagccgcagctgccgccgccgctgccgccgcaggtagtggagcaggcgctggaggagccggaggctacggagcgggagctggagcaggtgccggtgcaggtgctggcggcgcatctggaggctacggttcttacggatcgggagttgcagcaggtgccggtgcaggagctggtgttggtggtagcaggggagcaggtgttggcgctggtgttggtgctggttatggctccgcattgaattcaggagccggtgccggagcaggtgctggtgctggagctggtggtgctgcaggagctggtgctggtgcaggagcaggagctggcgctggagctgga

SEQ ID NO: 29 - DNA, 56 bp, synthetic construct
  misc_feature 1..56: note = primer
  source 1..56: mol_type = other DNA
taatgctcaaagatatatgccagccaggtgcacaagcattcacgtctaaatacgaa

SEQ ID NO: 30 - DNA, 20 bp, synthetic construct
  misc_feature 1..20: note = primer
  source 1..20: mol_type = other DNA
cagacatataagagctacga

SEQ ID NO: 31 - DNA, 21 bp, synthetic construct
  misc_feature 1..21: note = primer
  source 1..21: mol_type = other DNA
tgatattcgtcagtgtctgct

SEQ ID NO: 32 - DNA, 20 bp, synthetic construct
  misc_feature 1..20: note = primer
  source 1..20: mol_type = other DNA
tggtttgtccaaactcatca

SEQ ID NO: 33 - DNA, 20 bp, synthetic construct
  misc_feature 1..20: note = primer
  source 1..20: mol_type = other DNA
cacaatttgcataaaatgtc

SEQ ID NO: 34 - protein, 2136 aa, synthetic construct
  REGION 1..2136: note = synthetic
MKPIFLVLLVATSAYAAPSVTINQYSDNEIPRDIDDGKASSVISRAWDYVDDTDKSIAILNVQEILKDMASQGDYASQASAVAQTAGIIAHLSAGIPGDACAAANVINSYTDGVRSGNFAGFRQSLGPFFGHVGQNLNLINQLVINPGQLRYSVGPALGCAGGGRIYDFEAAWDAILASSDSSFLNEEYCIVKRLYNSRNSQSNNIAAYITAHLLPPVAQVFHQSAGSITDLLRGVGNGNDATGLVANAQRYIAQAFTSKYEAMAKADWYEDWKKNQGSFRETDLADTDEYQTDSNGTMFEKKTTRKKFEKDGSTMVNSDSGEDKIVRTFVVETDASGHEVIYEEDVVIKKVPGKRKKVSQANAKASAIAASVGAGVGAASVAGAGTGAGSGAAGGAGAGADAGAAAAAAAAAQAAAAAAAAAGSGAGAGRVGAYGPYGGLASAGAGGAGGAGGAGGYGGASVVYVGGGGAGAGAGSGAGAGSGAGAGAGSGAGAGGAGAAAGAGAGAGSGAGSGSGAGAGAGSGAGAGSGAGAGAGAGSGAAGGAGAGAGAGAGAAAAAAAAAEAAAAAAAAAAAAGSGAGAGGAGGYGAGAGAGAGAGAGGAAGAGGAGGAGGAGGYGGASAGAGGAGGAGGAGGYGGAGVVYVSAGGAGAGAGSGAGAGSGAGAGAGSGAGAGGAGAAAGAGAGAGSGAGSGSGAGAGAGSGAGAGSGAGAGAGAGSGAAGGAGAGAGAGAAAAAAAAAEAAAAAAAAAAAAGSGAGAGGAGGYGAGAGAGAGAGAGGASGGYGSYGSGVAAGAGAGAGVGGSRGAGVGAGVGAGYGSALNSGAGAGAGAGAGAGGAAGAGAGAGAGAGSGAAGGAGAGAGAGAAAAAAAAAEAAAAAAAAAAAAGGAGGYGAGAGAGAGAGAGTSAGAGGAGGAGGAGGYGGAGVVYVSAGGAGAGAGSGAGAGSGAGAGAGSGAGAGGAGAAAGAGAGAGSGAGSGSGAGAGAGSGAGAGSGAGAGAGAGSGAAGGAGAGAGAGAAAAAAAAAEAAAAAAAAAAAAGSGAGAGGAGGYGAGAGAGAGAGAGGASGGYGSYGSGVAAGAGAGAGVGGSRGAGVGAGVGAGYGSALNSGAGAGAGAGAGAGGAAGAGAGAGAGAGSGAAGGAGAGAGAGAAAAAAAAAEAAAAAAAAAAAAGGAGGYGAGAGAGAGAGAGTSAGAGGAGGAGGAGGYGGAGVVYVSAGGAGAGAGSGAGAGSGAGAGAGSGAGAGGAGAAAGAGAGAGSGAGSGSGAGAGAGSGAGAGSGAGAGAGAGSGAAGGAGAGAGAGAAAAAAAAAEAAAAAAAAAAAAGSGAGAGGAGGYGAGAGAGAGAGAGGASGGYGSYGSGVAAGAGAGAGVGGSRGAGVGAGVGAGYGSALNSGAGAGAGAGAGAGGAAGAGAGAGAGAGSGAAGGAGAGAGAGAAAAAAAAAEAAAAAAAAAAAAGGAGGYGAGAGAGAGAGAGTSAGAGGAGGAGGAGGYGGAGVVYVSAGGAGAGAGSGAGAGSGAGAGAGSGAGAGGAGAAAGAGAGAGSGAGSGSGAGAGAGSGAGAGSGAGAGAGAGSGAAGGAGAGAGAGAAAAAAAAAEAAAAAAAAAAAAGSGAGAGGAGGYGAGAGAGAGAGAGGASGGYGSYGSGVAAGAGAGAGVGGSRGAGVGAGVGAGYGSALNSGAGAGAGAGAGAGGAAGAGAGAGAGAGSGAAGGAGAGAGAGAAAAAAAAAEAAAAAAAAAAAAGGAGGYGAGAGAGAGAGAGTSVVYVSAGGAGAGAGSGAGAGSGAGAGAGSGAGAGGAGAAAGAGAGAGSGAGSGSGAGAGAGSGAVAGSGAGSGAAGGAGAGAGAGAAAAAAAAAEAAAAAAAAAAAAGSGAGAGGAGGYGAGAGAGAGAGVGGAGGAGGAGGAGGAGGYGGAGVVYVSAGGAGAGAGSGAGAGSGAGAGAGSGAGAGGAGAAAGAGAGAGSGAGSGSGAGAGAGSGAVAGSGAGSGAAGGAGAGAGAGAAAAAAAAAEAAAAAAAAAAAAGSGAGAGGAGGYGAGAGAGAGAGAGGASGGYGSYGSGVAAGAGAGAGVGGSRGAGVGAGVGAGYGSALNSGAGAGAGAGAGAGGAAGAGAGAGAGAGAGAGLEHHHHHH